European Patent Application EP 4 455 294 A1, published October 30, 2024. Title: 신규한 프로모터 및 이의 이용. Applicant: 주식회사 툴젠. Application KR. The sequence listing filed with the application follows.

SEQUENCE LISTING (40 sequences)

SEQ ID NO: 1 - DNA, 900 bp, synthetic construct
  source 1..900: mol_type = other DNA
tgagagctcagccctgtaaccaggccttgccggagccactgatgcctggtcttctgtgcctttactccaaacaccccccagcccaagccacccacttgttctcaagtctgaagaagcccctcacccctctactccaggctgtgttcagggcttggggctggtggagggaggggcctgaaattccagtgtgaaaggctgagatgggcccgaggcccctggcctatgtccaagccatttcccctctcaccagcctctccctggggagccagtcagctaggaaggaatgagggctccccaggcccacccccagttcctgagctcatctgggctgcagggctggcgggacagcagcgtggactcagtctcctagggatttcccaactctcccgcccgcttgctgcatctggacaccctgcctcaggccctcatctccactggtcagcaggtgacctttgcccagcgccctgggtcctcagtgcctgctgccctggagatgatataaaacaggtcagaaccctcctgcctgtctgctcagttcatccctagaggcagctgctccaggtaatgccctctggggaggggaaagaggaggggaggaggatgaagaggggcaagaggagctccctgcccagcccagccagcaagcctggagaagcacttgctagagctaaggaagcctcggagctggacgggtgccccccacccctcatcataacctgaagaacatggaggcccgggaggggtgtcacttgcccaaagctacacagggggtggggctggaagtggctccaagtgcaggttcccccctcattcttcaggcttagggctggaggaagccttagacagcccagtcctaccccagacagggaaactgaggcctggagagggccagaaatcacc

SEQ ID NO: 2 - DNA, 440 bp, synthetic construct
  source 1..440: mol_type = other DNA
cgccctgggtcctcagtgcctgctgccctggagatgatataaaacaggtcagaaccctcctgcctgtctgctcagttcatccctagaggcagctgctccaggtaatgccctctggggaggggaaagaggaggggaggaggatgaagaggggcaagaggagctccctgcccagcccagccagcaagcctggagaagcacttgctagagctaaggaagcctcggagctggacgggtgccccccacccctcatcataacctgaagaacatggaggcccgggaggggtgtcacttgcccaaagctacacagggggtggggctggaagtggctccaagtgcaggttcccccctcattcttcaggcttagggctggaggaagccttagacagcccagtcctaccccagacagggaaactgaggcctggagagggccagaaatcacc

SEQ ID NO: 3 - DNA, 589 bp, synthetic construct
  source 1..589: mol_type = other DNA
tcctgagctcatctgggctgcagggctggcgggacagcagcgtggactcagtctcctagggatttcccaactctcccgcccgcttgctgcatctggacaccctgcctcaggccctcatctccactggtcagcaggtgacctttgcccagcgccctgggtcctcagtgcctgctgccctggagatgatataaaacaggtcagaaccctcctgcctgtctgctcagttcatccctagaggcagctgctccaggtaatgccctctggggaggggaaagaggaggggaggaggatgaagaggggcaagaggagctccctgcccagcccagccagcaagcctggagaagcacttgctagagctaaggaagcctcggagctggacgggtgccccccacccctcatcataacctgaagaacatggaggcccgggaggggtgtcacttgcccaaagctacacagggggtggggctggaagtggctccaagtgcaggttcccccctcattcttcaggcttagggctggaggaagccttagacagcccagtcctaccccagacagggaaactgaggcctggagagggccagaaatcacc

SEQ ID NO: 4 - DNA, 167 bp, synthetic construct
  source 1..167: mol_type = other DNA
cgccctgggtcctcagtgcctgctgccctggagatgatataaaacaggtcagaaccctcctgcctgtctgctcagttcatccctagaggcagctgctccaggtaatgccctctggggaggggaaagaggaggggaggaggatgaagaggggcaagaggagctccctg

SEQ ID NO: 5 - DNA, 316 bp, synthetic construct
  source 1..316: mol_type = other DNA
tcctgagctcatctgggctgcagggctggcgggacagcagcgtggactcagtctcctagggatttcccaactctcccgcccgcttgctgcatctggacaccctgcctcaggccctcatctccactggtcagcaggtgacctttgcccagcgccctgggtcctcagtgcctgctgccctggagatgatataaaacaggtcagaaccctcctgcctgtctgctcagttcatccctagaggcagctgctccaggtaatgccctctggggaggggaaagaggaggggaggaggatgaagaggggcaagaggagctccctg

SEQ ID NO: 6 - DNA, 1000 bp, synthetic construct
  source 1..1000: mol_type = other DNA
tgcccagctacggcagaggagactgttgggatcacaggtggaggtcagtgtgggggcatgtaaccttcactctgccccctcccaccccacttcctccgttgctccacagtggcaccacagattccccattccattctactggaaggctttcaggtggcttctgtgaaggagcctgtcactggctctaggctgtaaagcaggcctgaggtccaaggcttgtcccctgtcttttcctgtctcaccgacctcatctaggtgagccggtagctgatcccttggtggcggaggtggccgtgaaaagcatgggcaatctcagagggatttctcaactcctctggcagatggctgcatggccttcctgcctcaggctctggtctggactgctcagcaggtgacctttgcccagctcactgggccttctgtgcccgctgtcccatcctggagccaatataaaacaggtcacagccctccccgcttgcctgctcagttttatccctagaagcagctagctactccaggtaatgcccctggggaggagaggaaggaagggaagaaacaaagagctggagggagaagctctcaccacccagccatctagcccacagaaggcttgggactcatggtctccacccttgggttcctggtgtggggggggctagaagctggggaaagggaggctatgggccaaaagccttgcactgggtagtggcagagctgcctgcaattgggtcatgctgtcccttgtttagcttgctctgagctattagaagcctttggtatccatgcctacccaggactgaaaaaactgagtcctagcgaggaaaagaaacctattgtttctcagcatattagagtagatgtcccgttctgcagagtatttctatactccaccttccaggttcccccctcattcttcaggcttagggctggaggaagccttagacagcccagtcctaccccagacagggaaactgaggcctggagagggccagaaatcacc

SEQ ID NO: 7 - DNA, 900 bp, synthetic construct
  source 1..900: mol_type = other DNA
caaagacacacagcatgttggctggactggacggagatcagtccagaccgcaggtgccttgatgttcagtctggtgggttttctgctccatcccacccacctccctttgggcctcgatccctcgcccctcaccagtcccccttctgagagcccgtattagcagggagccggcccctactccttctggcagacccagctaaggttctaccttaggggccacgccacctccccagggaggggtccagaggcatggggacctggggtgcccctcacaggacacttccttgcaggaacagaggtgccatgcagccccgggtactccttgttgttgccctcctggcgctcctggcctctgcccgtaagcacttggtgggactgggctgggggcagggtggaggcaacttggggatcccagtcccaatgggtggtcaagcaggagcccagggctcgtccagaggccgatccaccccactcagccctgctctttcctcaggagcttcagaggccgaggatgcctcccttctcagcttcatgcagggttacatgaagcacgccaccaagaccgccaaggatgcactgagcagcgtgcaggagtcccaggtggcccagcaggccaggtacacccgctggcctccctccccatcccccctgccagctgcctccattcccacccgcccctgccctggtgagatcccaacaatggaatggaggtgctccagcctcccctgggcctgtgcctcttcagcctcctctttcctcacagggcctttgtcaggctgctgcgggagagatgacagagttgagactgcattcctcccaggtccctcctttctccccggagcagtcctagggcgtgccgttttagccctcatttccattttcctttcctttccctttctt

SEQ ID NO: 8 - DNA, 1000 bp, synthetic construct
  source 1..1000: mol_type = other DNA
caaagacacacagaccacttggggggctgggtctactgtagttctctatctaatatcagtgggagaaaggcttgggattcatgacccaggagtcatggcattctcaaggggaggacctagatgtggcagatccacagtaccttctcacgagatgctttcccacaggtacgtaggtgccatgcagccccggacgctcctcactgtggccctcttggctctcctggcatctgcccgtaagatggtgggagtggggctgggtttcagtgggagctggtcagggggccctgccctgagaagtggtggctgggcaggagctgagggctggcgtggcccaactctgctctctcgcaggagctgaagaggtagagggatccttgctgctgggctctgtacagggctacatggaacaagcctccaagacggtccaggatgcgctaagtagcgtgcaggagtccgatatagctgtggtggccaggtaggcacactggcctcctttcctgtgtcttctcctctcatgccctggtgctaagaccctagcacagagactgtggtccaccaagtttaccagggcctgggacccgcccgagcctctggtccctcatgaggcctttcggtactgtgaccaagatgacaggcagggcaagcagccttctcctatcttctctgcttttcctcagagcagcctgaggggcatttagcctcgctgcaggttttctcctctgggtcctgcgcacacgatgggaggcctacctgctctggtttctgcctgtatgcagggggtagtggtgggaagtgaggtgggaagttgggggttagagggtgggagtctgccctgtttctatccctgggctcagtctgaggtaggcatcttgcccactatgaaatatcaccccctggccaatggctttggctgacatttgatagtttagttgcctatgtagcaaaagatgttgacagtctctatccccagaacaggctgtggggaggatattagatactc

SEQ ID NO: 9 - DNA, 629 bp, Homo sapiens
  source 1..629: mol_type = genomic DNA
gtaatgccctctggggaggggaaagaggaggggaggaggatgaagaggggcaagaggagctccctgcccagcccagccagcaagcctggagaagcacttgctagagctaaggaagcctcggagctggacgggtgccccccacccctcatcataacctgaagaacatggaggcccgggaggggtgtcacttgcccaaagctacacagggggtggggctggaagtggctccaagtgcaggttcccccctcattcttcaggcttagggctggaggaagccttagacagcccagtcctaccccagacagggaaactgaggcctggagagggccagaaatcacccaaagacacacagcatgttggctggactggacggagatcagtccagaccgcaggtgccttgatgttcagtctggtgggttttctgctccatcccacccacctccctttgggcctcgatccctcgcccctcaccagtcccccttctgagagcccgtattagcagggagccggcccctactccttctggcagacccagctaaggttctaccttaggggccacgccacctccccagggaggggtccagaggcatggggacctggggtgcccctcacaggacacttccttgcag

SEQ ID NO: 10 - DNA, 532 bp, synthetic construct
  source 1..532: mol_type = other DNA
gtaatgcccctggggaggagaggaaggaagggaagaaacaaagagctggagggagaagctctcaccacccagccatctagcccacagaaggcttgggactcatggtctccacccttgggttcctggtgtggggggggctagaagctggggaaagggaggctatgggccaaaagccttgcactgggtagtggcagagctgcctgcaattgggtcatgctgtcccttgtttagcttgctctgagctattagaagcctttggtatccatgcctacccaggactgaaaaaactgagtcctagcgaggaaaagaaacctattgtttctcagcatattagagtagatgtcccgttctgcagagtatttctatactccaccttccaccccacttggggggctgggtctactgtagttctctatctaatatcagtgggagaaaggcttgggattcatgacccaggagtcatggcattctcaaggggaggacctagatgtggcagatccacagtaccttctcacgagatgctttcccacag

SEQ ID NO: 11 - DNA, 438 bp, synthetic construct
  source 1..438: mol_type = other DNA
gtgggtgggggaggctagaagctgaggaaagggaggccactgggccaaaaaagccttgcactgggtagtggcagagctgatgggaactgggtcatgctgccccttgttcgtcttgctctgagctattagaagcctttgatatccgtgcctaccccagactgaaaagcctgaagcctagagagaaaaagaaacctgttgtttctccatatattggggcagaggctgggtagatgttctgctttgcagaggattcccacattccaccttccagcccccttggggtgggtctgggtcttctatagttctctctccgagagctgatatcagtaggagaaaggcttggggattcatgacccaggcaggggccgtggtgttctccagggaagggcttagatgtggcagatccacaataccctctcacaagatggtctcccgcag

SEQ ID NO: 12-16 - skipped (5 entries)

SEQ ID NO: 17 - DNA, 12 bp, synthetic construct
  source 1..12: mol_type = other DNA
aggtgacctttc

SEQ ID NO: 18-24 - skipped (7 entries)

SEQ ID NO: 25 - DNA, 40 bp, synthetic construct
  source 1..40: mol_type = other DNA
ggagagggccagaaatcacccaaagacacacagcatgttg

SEQ ID NO: 26 - DNA, 25 bp, synthetic construct
  source 1..25: mol_type = other DNA
ctgacctcttctcttcctcccacag

SEQ ID NO: 27 - DNA, 225 bp, synthetic construct
  source 1..225: mol_type = other DNA
ctgtgccttctagttgccagccatctgttgtttgcccctcccccgtgccttccttgaccctggaaggtgccactcccactgtcctttcctaataaaatgaggaaattgcatcgcattgtctgagtaggtgtcattctattctggggggtggggtggggcaggacagcaagggggaggattgggaagacaatagcaggcatgctggggatgcggtgggctctatgg

SEQ ID NO: 28 - DNA, 726 bp, synthetic construct
  source 1..726: mol_type = other DNA
atggtgagcaagggcgaggagctgttcaccggggtggtgcccatcctggtcgagctggacggcgacgtaaacggccacaagttcagcgtgtccggcgagggcgagggcgatgccacctacggcaagctgaccctgaagttcatctgcaccaccggcaagctgcccgtgccctggcccaccctcgtgaccaccctgacctacggcgtgcagtgcttcagccgctaccccgaccacatgaagcagcacgacttcttcaagtccgccatgcccgaaggctacgtccaggagcgcaccatcttcttcaaggacgacggcaactacaagacccgcgccgaggtgaagttcgagggcgacaccctggtgaaccgcatcgagctgaagggcatcgacttcaaggaggacggcaacatcctggggcacaagctggagtacaactacaacagccacaacgtctatatcatggccgacaagcagaagaacggcatcaaggtgaacttcaagatccgccacaacatcgaggacggcagcgtgcagctcgccgaccactaccagcagaacacccccatcggcgacggccccgtgctgctgcccgacaaccactacctgagcacccagtccgccctgagcaaagaccccaacgagaagcgcgatcacatggtcctgctggagttcgtgaccgccgccgggatcactctcggcatggacgagctgtacaagtccggataa

SEQ ID NO: 29 - DNA, 2790 bp, synthetic construct
  source 1..2790: mol_type = other DNA
tgagagctcagccctgtaaccaggccttgccggagccactgatgcctggtcttctgtgcctttactccaaacaccccccagcccaagccacccacttgttctcaagtctgaagaagcccctcacccctctactccaggctgtgttcagggcttggggctggtggagggaggggcctgaaattccagtgtgaaaggctgagatgggcccgaggcccctggcctatgtccaagccatttcccctctcaccagcctctccctggggagccagtcagctaggaaggaatgagggctccccaggcccacccccagttcctgagctcatctgggctgcagggctggcgggacagcagcgtggactcagtctcctagggatttcccaactctcccgcccgcttgctgcatctggacaccctgcctcaggccctcatctccactggtcagcaggtgacctttgcccagcgccctgggtcctcagtgcctgctgccctggagatgatataaaacaggtcagaaccctcctgcctgtctgctcagttcatccctagaggcagctgctccaggtaatgccctctggggaggggaaagaggaggggaggaggatgaagaggggcaagaggagctccctgcccagcccagccagcaagcctggagaagcacttgctagagctaaggaagcctcggagctggacgggtgccccccacccctcatcataacctgaagaacatggaggcccgggaggggtgtcacttgcccaaagctacacagggggtggggctggaagtggctccaagtgcaggttcccccctcattcttcaggcttagggctggaggaagccttagacagcccagtcctaccccagacagggaaactgaggcctggagagggccagaaatcaccctgacctcttctcttcctcccacagtatggtgagcaagggcgaggagctgttcaccggggtggtgcccatcctggtcgagctggacggcgacgtaaacggccacaagttcagcgtgtccggcgagggcgagggcgatgccacctacggcaagctgaccctgaagttcatctgcaccaccggcaagctgcccgtgccctggcccaccctcgtgaccaccctgacctacggcgtgcagtgcttcagccgctaccccgaccacatgaagcagcacgacttcttcaagtccgccatgcccgaaggctacgtccaggagcgcaccatcttcttcaaggacgacggcaactacaagacccgcgccgaggtgaagttcgagggcgacaccctggtgaaccgcatcgagctgaagggcatcgacttcaaggaggacggcaacatcctggggcacaagctggagtacaactacaacagccacaacgtctatatcatggccgacaagcagaagaacggcatcaaggtgaacttcaagatccgccacaacatcgaggacggcagcgtgcagctcgccgaccactaccagcagaacacccccatcggcgacggccccgtgctgctgcccgacaaccactacctgagcacccagtccgccctgagcaaagaccccaacgagaagcgcgatcacatggtcctgctggagttcgtgaccgccgccgggatcactctcggcatggacgagctgtacaagtccggataactcagatctcgagctgtgccttctagttgccagccatctgttgtttgcccctcccccgtgccttccttgaccctggaaggtgccactcccactgtcctttcctaataaaatgaggaaattgcatcgcattgtctgagtaggtgtcattctattctggggggtggggtggggcaggacagcaagggggaggattgggaagacaatagcaggcatgctggggatgcggtgggctctatggcaaagacacacagcatgttggctggactggacggagatcagtccagaccgcaggtgccttgatgttcagtctggtgggttttctgctccatcccacccacctccctttgggcctcgatccctcgcccctcaccagtcccccttctgagagcccgtattagcagggagccggcccctactccttctggcagacccagctaaggttctaccttaggggccacgccacctccccagggaggggtccagaggcatggggacctggggtgcccctcacaggacacttccttgcaggaacagaggtgccatgcagccccgggtactccttgttgttgccctcctggcgctcctggcctctgcccgtaagcacttggtgggactgggctgggggcagggtggaggcaacttggggatcccagtcccaatgggtggtcaagcaggagcccagggctcgtccagaggccgatccaccccactcagccctgctctttcctcaggagcttcagaggccgaggatgcctcccttctcagcttcatgcagggttacatgaagcacgccaccaagaccgccaaggatgcactgagcagcgtgcaggagtcccaggtggcccagcaggccaggtacacccgctggcctccctccccatcccccctgccagctgcctccattcccacccgcccctgccctggtgagatcccaacaatggaatggaggtgctccagcctcccctgggcctgtgcctcttcagcctcctctttcctcacagggcctttgtcaggctgctgcgggagagatgacagagttgagactgcattcctcccaggtccctcctttctccccggagcagtcctagggcgtgccgttttagccctcatttccattttcctttcctttccctttctt

SEQ ID NO: 30 - DNA, 1890 bp, synthetic construct
  source 1..1890: mol_type = other DNA
tgagagctcagccctgtaaccaggccttgccggagccactgatgcctggtcttctgtgcctttactccaaacaccccccagcccaagccacccacttgttctcaagtctgaagaagcccctcacccctctactccaggctgtgttcagggcttggggctggtggagggaggggcctgaaattccagtgtgaaaggctgagatgggcccgaggcccctggcctatgtccaagccatttcccctctcaccagcctctccctggggagccagtcagctaggaaggaatgagggctccccaggcccacccccagttcctgagctcatctgggctgcagggctggcgggacagcagcgtggactcagtctcctagggatttcccaactctcccgcccgcttgctgcatctggacaccctgcctcaggccctcatctccactggtcagcaggtgacctttgcccagcgccctgggtcctcagtgcctgctgccctggagatgatataaaacaggtcagaaccctcctgcctgtctgctcagttcatccctagaggcagctgctccaggtaatgccctctggggaggggaaagaggaggggaggaggatgaagaggggcaagaggagctccctgcccagcccagccagcaagcctggagaagcacttgctagagctaaggaagcctcggagctggacgggtgccccccacccctcatcataacctgaagaacatggaggcccgggaggggtgtcacttgcccaaagctacacagggggtggggctggaagtggctccaagtgcaggttcccccctcattcttcaggcttagggctggaggaagccttagacagcccagtcctaccccagacagggaaactgaggcctggagagggccagaaatcaccctgacctcttctcttcctcccacagtatggtgagcaagggcgaggagctgttcaccggggtggtgcccatcctggtcgagctggacggcgacgtaaacggccacaagttcagcgtgtccggcgagggcgagggcgatgccacctacggcaagctgaccctgaagttcatctgcaccaccggcaagctgcccgtgccctggcccaccctcgtgaccaccctgacctacggcgtgcagtgcttcagccgctaccccgaccacatgaagcagcacgacttcttcaagtccgccatgcccgaaggctacgtccaggagcgcaccatcttcttcaaggacgacggcaactacaagacccgcgccgaggtgaagttcgagggcgacaccctggtgaaccgcatcgagctgaagggcatcgacttcaaggaggacggcaacatcctggggcacaagctggagtacaactacaacagccacaacgtctatatcatggccgacaagcagaagaacggcatcaaggtgaacttcaagatccgccacaacatcgaggacggcagcgtgcagctcgccgaccactaccagcagaacacccccatcggcgacggccccgtgctgctgcccgacaaccactacctgagcacccagtccgccctgagcaaagaccccaacgagaagcgcgatcacatggtcctgctggagttcgtgaccgccgccgggatcactctcggcatggacgagctgtacaagtccggataactcagatctcgagctgtgccttctagttgccagccatctgttgtttgcccctcccccgtgccttccttgaccctggaaggtgccactcccactgtcctttcctaataaaatgaggaaattgcatcgcattgtctgagtaggtgtcattctattctggggggtggggtggggcaggacagcaagggggaggattgggaagacaatagcaggcatgctggggatgcggtgggctctatgg

SEQ ID NO: 31 - DNA, 21 bp, synthetic construct
  source 1..21: mol_type = other DNA
ggaacccctagtgatggagtt

SEQ ID NO: 32 - DNA, 16 bp, synthetic construct
  source 1..16: mol_type = other DNA
cggcctcagtgagcga

SEQ ID NO: 33 - DNA, 1386 bp, synthetic construct
  source 1..1386: mol_type = other DNA
atgcagcgcgtgaacatgatcatggccgagtctcctggcctgatcaccatctgcctgctgggctacctgctgagcgccgagtgcaccgtgtttctggaccacgagaacgccaacaagatcctgaaccggcccaagcggtacaacagcggcaagctggaagagttcgtgcagggcaacctggaacgcgagtgcatggaagagaagtgcagctttgaagaggccagagaggtgttcgagaacaccgagcggaccaccgagttctggaagcagtatgttgatggagatcagtgtgagtccaatccatgtttaaatggcggcagttgcaaggatgacattaattcctatgaatgttggtgtccctttggcttcgagggcaagaactgtgaattagatgtaacatgtaacattaagaatggcagatgcgagcagttttgtaaaaatagtgctgataacaaggtggtttgctcctgtactgagggatatcgacttgcagaaaaccagaagtcctgcgagcccgccgtgcctttcccatgtggaagagtgtccgtgtcccagaccagcaagctgaccagagccgagacagtgttccccgacgtggactacgtgaacagcaccgaggccgagacaatcctggacaacatcacccagagcacccagtccttcaacgacttcaccagagtcgtgggcggcgaggatgccaagcctggacagttcccgtggcaggtggtgctgaacggaaaggtggacgccttttgcggcggcagcatcgtgaatgaaaaatggattgtaactgctgcccactgtgttgaaactggtgttaaaattacagttgtcgcaggtgaacataacatcgaggaaaccgaacatacagagcaaaagcgaaatgtgattcgaattattcctcaccacaactacaatgcagctattaataagtacaaccatgacattgcccttctggaactggacgaacccttagtgctaaacagctacgttacacctatttgcattgctgacaaagagtacaccaacatctttctgaagttcggcagcggctacgtgtccggctggggcagagtgtttcacaagggcagatccgctctggtgctgcagtacctgagagtgcctctggtggaccgggccacctgtctgagaagcaccaagttcaccatctacaacaacatgttctgcgccggctttcacgagggcggcagagatagctgtcagggcgattctggcggccctcacgtgacagaggtggaaggcaccagctttctgaccggcatcatcagctggggcgaggaatgcgccatgaaggggaagtacggcatctacaccaaggtgtccagatacgtgaactggatcaaagaaaagaccaagctgacatga

SEQ ID NO: 34 - DNA, 3436 bp, synthetic construct
  source 1..3436: mol_type = other DNA
tgagagctcagccctgtaaccaggccttgccggagccactgatgcctggtcttctgtgcctttactccaaacaccccccagcccaagccacccacttgttctcaagtctgaagaagcccctcacccctctactccaggctgtgttcagggcttggggctggtggagggaggggcctgaaattccagtgtgaaaggctgagatgggcccgaggcccctggcctatgtccaagccatttcccctctcaccagcctctccctggggagccagtcagctaggaaggaatgagggctccccaggcccacccccagttcctgagctcatctgggctgcagggctggcgggacagcagcgtggactcagtctcctagggatttcccaactctcccgcccgcttgctgcatctggacaccctgcctcaggccctcatctccactggtcagcaggtgacctttgcccagcgccctgggtcctcagtgcctgctgccctggagatgatataaaacaggtcagaaccctcctgcctgtctgctcagttcatccctagaggcagctgctccaggtaatgccctctggggaggggaaagaggaggggaggaggatgaagaggggcaagaggagctccctgcccagcccagccagcaagcctggagaagcacttgctagagctaaggaagcctcggagctggacgggtgccccccacccctcatcataacctgaagaacatggaggcccgggaggggtgtcacttgcccaaagctacacagggggtggggctggaagtggctccaagtgcaggttcccccctcattcttcaggcttagggctggaggaagccttagacagcccagtcctaccccagacagggaaactgaggcctggagagggccagaaatcaccctgacctcttctcttcctcccacagatgcagcgcgtgaacatgatcatggccgagtctcctggcctgatcaccatctgcctgctgggctacctgctgagcgccgagtgcaccgtgtttctggaccacgagaacgccaacaagatcctgaaccggcccaagcggtacaacagcggcaagctggaagagttcgtgcagggcaacctggaacgcgagtgcatggaagagaagtgcagctttgaagaggccagagaggtgttcgagaacaccgagcggaccaccgagttctggaagcagtatgttgatggagatcagtgtgagtccaatccatgtttaaatggcggcagttgcaaggatgacattaattcctatgaatgttggtgtccctttggcttcgagggcaagaactgtgaattagatgtaacatgtaacattaagaatggcagatgcgagcagttttgtaaaaatagtgctgataacaaggtggtttgctcctgtactgagggatatcgacttgcagaaaaccagaagtcctgcgagcccgccgtgcctttcccatgtggaagagtgtccgtgtcccagaccagcaagctgaccagagccgagacagtgttccccgacgtggactacgtgaacagcaccgaggccgagacaatcctggacaacatcacccagagcacccagtccttcaacgacttcaccagagtcgtgggcggcgaggatgccaagcctggacagttcccgtggcaggtggtgctgaacggaaaggtggacgccttttgcggcggcagcatcgtgaatgaaaaatggattgtaactgctgcccactgtgttgaaactggtgttaaaattacagttgtcgcaggtgaacataacatcgaggaaaccgaacatacagagcaaaagcgaaatgtgattcgaattattcctcaccacaactacaatgcagctattaataagtacaaccatgacattgcccttctggaactggacgaacccttagtgctaaacagctacgttacacctatttgcattgctgacaaagagtacaccaacatctttctgaagttcggcagcggctacgtgtccggctggggcagagtgtttcacaagggcagatccgctctggtgctgcagtacctgagagtgcctctggtggaccgggccacctgtctgagaagcaccaagttcaccatctacaacaacatgttctgcgccggctttcacgagggcggcagagatagctgtcagggcgattctggcggccctcacgtgacagaggtggaaggcaccagctttctgaccggcatcatcagctggggcgaggaatgcgccatgaaggggaagtacggcatctacaccaaggtgtccagatacgtgaactggatcaaagaaaagaccaagctgacatgactgtgccttctagttgccagccatctgttgtttgcccctcccccgtgccttccttgaccctggaaggtgccactcccactgtcctttcctaataaaatgaggaaattgcatcgcattgtctgagtaggtgtcattctattctggggggtggggtggggcaggacagcaagggggaggattgggaagacaatagcaggcatgctggggatgcggtgggctctatggcaaagacacacagcatgttggctggactggacggagatcagtccagaccgcaggtgccttgatgttcagtctggtgggttttctgctccatcccacccacctccctttgggcctcgatccctcgcccctcaccagtcccccttctgagagcccgtattagcagggagccggcccctactccttctggcagacccagctaaggttctaccttaggggccacgccacctccccagggaggggtccagaggcatggggacctggggtgcccctcacaggacacttccttgcaggaacagaggtgccatgcagccccgggtactccttgttgttgccctcctggcgctcctggcctctgcccgtaagcacttggtgggactgggctgggggcagggtggaggcaacttggggatcccagtcccaatgggtggtcaagcaggagcccagggctcgtccagaggccgatccaccccactcagccctgctctttcctcaggagcttcagaggccgaggatgcctcccttctcagcttcatgcagggttacatgaagcacgccaccaagaccgccaaggatgcactgagcagcgtgcaggagtcccaggtggcccagcaggccaggtacacccgctggcctccctccccatcccccctgccagctgcctccattcccacccgcccctgccctggtgagatcccaacaatggaatggaggtgctccagcctcccctgggcctgtgcctcttcagcctcctctttcctcacagggcctttgtcaggctgctgcgggagagatgacagagttgagactgcattcctcccaggtccctcctttctccccggagcagtcctagggcgtgccgttttagccctcatttccattttcctttcctttccctttctt

SEQ ID NO: 35 - DNA, 2536 bp, synthetic construct
  source 1..2536: mol_type = other DNA
tgagagctcagccctgtaaccaggccttgccggagccactgatgcctggtcttctgtgcctttactccaaacaccccccagcccaagccacccacttgttctcaagtctgaagaagcccctcacccctctactccaggctgtgttcagggcttggggctggtggagggaggggcctgaaattccagtgtgaaaggctgagatgggcccgaggcccctggcctatgtccaagccatttcccctctcaccagcctctccctggggagccagtcagctaggaaggaatgagggctccccaggcccacccccagttcctgagctcatctgggctgcagggctggcgggacagcagcgtggactcagtctcctagggatttcccaactctcccgcccgcttgctgcatctggacaccctgcctcaggccctcatctccactggtcagcaggtgacctttgcccagcgccctgggtcctcagtgcctgctgccctggagatgatataaaacaggtcagaaccctcctgcctgtctgctcagttcatccctagaggcagctgctccaggtaatgccctctggggaggggaaagaggaggggaggaggatgaagaggggcaagaggagctccctgcccagcccagccagcaagcctggagaagcacttgctagagctaaggaagcctcggagctggacgggtgccccccacccctcatcataacctgaagaacatggaggcccgggaggggtgtcacttgcccaaagctacacagggggtggggctggaagtggctccaagtgcaggttcccccctcattcttcaggcttagggctggaggaagccttagacagcccagtcctaccccagacagggaaactgaggcctggagagggccagaaatcaccctgacctcttctcttcctcccacagatgcagcgcgtgaacatgatcatggccgagtctcctggcctgatcaccatctgcctgctgggctacctgctgagcgccgagtgcaccgtgtttctggaccacgagaacgccaacaagatcctgaaccggcccaagcggtacaacagcggcaagctggaagagttcgtgcagggcaacctggaacgcgagtgcatggaagagaagtgcagctttgaagaggccagagaggtgttcgagaacaccgagcggaccaccgagttctggaagcagtatgttgatggagatcagtgtgagtccaatccatgtttaaatggcggcagttgcaaggatgacattaattcctatgaatgttggtgtccctttggcttcgagggcaagaactgtgaattagatgtaacatgtaacattaagaatggcagatgcgagcagttttgtaaaaatagtgctgataacaaggtggtttgctcctgtactgagggatatcgacttgcagaaaaccagaagtcctgcgagcccgccgtgcctttcccatgtggaagagtgtccgtgtcccagaccagcaagctgaccagagccgagacagtgttccccgacgtggactacgtgaacagcaccgaggccgagacaatcctggacaacatcacccagagcacccagtccttcaacgacttcaccagagtcgtgggcggcgaggatgccaagcctggacagttcccgtggcaggtggtgctgaacggaaaggtggacgccttttgcggcggcagcatcgtgaatgaaaaatggattgtaactgctgcccactgtgttgaaactggtgttaaaattacagttgtcgcaggtgaacataacatcgaggaaaccgaacatacagagcaaaagcgaaatgtgattcgaattattcctcaccacaactacaatgcagctattaataagtacaaccatgacattgcccttctggaactggacgaacccttagtgctaaacagctacgttacacctatttgcattgctgacaaagagtacaccaacatctttctgaagttcggcagcggctacgtgtccggctggggcagagtgtttcacaagggcagatccgctctggtgctgcagtacctgagagtgcctctggtggaccgggccacctgtctgagaagcaccaagttcaccatctacaacaacatgttctgcgccggctttcacgagggcggcagagatagctgtcagggcgattctggcggccctcacgtgacagaggtggaaggcaccagctttctgaccggcatcatcagctggggcgaggaatgcgccatgaaggggaagtacggcatctacaccaaggtgtccagatacgtgaactggatcaaagaaaagaccaagctgacatgactgtgccttctagttgccagccatctgttgtttgcccctcccccgtgccttccttgaccctggaaggtgccactcccactgtcctttcctaataaaatgaggaaattgcatcgcattgtctgagtaggtgtcattctattctggggggtggggtggggcaggacagcaagggggaggattgggaagacaatagcaggcatgctggggatgcggtgggctctatgg

SEQ ID NO: 36 - DNA, 2076 bp, synthetic construct
  source 1..2076: mol_type = other DNA
cgccctgggtcctcagtgcctgctgccctggagatgatataaaacaggtcagaaccctcctgcctgtctgctcagttcatccctagaggcagctgctccaggtaatgccctctggggaggggaaagaggaggggaggaggatgaagaggggcaagaggagctccctgcccagcccagccagcaagcctggagaagcacttgctagagctaaggaagcctcggagctggacgggtgccccccacccctcatcataacctgaagaacatggaggcccgggaggggtgtcacttgcccaaagctacacagggggtggggctggaagtggctccaagtgcaggttcccccctcattcttcaggcttagggctggaggaagccttagacagcccagtcctaccccagacagggaaactgaggcctggagagggccagaaatcaccctgacctcttctcttcctcccacagatgcagcgcgtgaacatgatcatggccgagtctcctggcctgatcaccatctgcctgctgggctacctgctgagcgccgagtgcaccgtgtttctggaccacgagaacgccaacaagatcctgaaccggcccaagcggtacaacagcggcaagctggaagagttcgtgcagggcaacctggaacgcgagtgcatggaagagaagtgcagctttgaagaggccagagaggtgttcgagaacaccgagcggaccaccgagttctggaagcagtatgttgatggagatcagtgtgagtccaatccatgtttaaatggcggcagttgcaaggatgacattaattcctatgaatgttggtgtccctttggcttcgagggcaagaactgtgaattagatgtaacatgtaacattaagaatggcagatgcgagcagttttgtaaaaatagtgctgataacaaggtggtttgctcctgtactgagggatatcgacttgcagaaaaccagaagtcctgcgagcccgccgtgcctttcccatgtggaagagtgtccgtgtcccagaccagcaagctgaccagagccgagacagtgttccccgacgtggactacgtgaacagcaccgaggccgagacaatcctggacaacatcacccagagcacccagtccttcaacgacttcaccagagtcgtgggcggcgaggatgccaagcctggacagttcccgtggcaggtggtgctgaacggaaaggtggacgccttttgcggcggcagcatcgtgaatgaaaaatggattgtaactgctgcccactgtgttgaaactggtgttaaaattacagttgtcgcaggtgaacataacatcgaggaaaccgaacatacagagcaaaagcgaaatgtgattcgaattattcctcaccacaactacaatgcagctattaataagtacaaccatgacattgcccttctggaactggacgaacccttagtgctaaacagctacgttacacctatttgcattgctgacaaagagtacaccaacatctttctgaagttcggcagcggctacgtgtccggctggggcagagtgtttcacaagggcagatccgctctggtgctgcagtacctgagagtgcctctggtggaccgggccacctgtctgagaagcaccaagttcaccatctacaacaacatgttctgcgccggctttcacgagggcggcagagatagctgtcagggcgattctggcggccctcacgtgacagaggtggaaggcaccagctttctgaccggcatcatcagctggggcgaggaatgcgccatgaaggggaagtacggcatctacaccaaggtgtccagatacgtgaactggatcaaagaaaagaccaagctgacatgactgtgccttctagttgccagccatctgttgtttgcccctcccccgtgccttccttgaccctggaaggtgccactcccactgtcctttcctaataaaatgaggaaattgcatcgcattgtctgagtaggtgtcattctattctggggggtggggtggggcaggacagcaagggggaggattgggaagacaatagcaggcatgctggggatgcggtgggctctatgg

SEQ ID NO: 37 - DNA, 2225 bp, synthetic construct
  source 1..2225: mol_type = other DNA
tcctgagctcatctgggctgcagggctggcgggacagcagcgtggactcagtctcctagggatttcccaactctcccgcccgcttgctgcatctggacaccctgcctcaggccctcatctccactggtcagcaggtgacctttgcccagcgccctgggtcctcagtgcctgctgccctggagatgatataaaacaggtcagaaccctcctgcctgtctgctcagttcatccctagaggcagctgctccaggtaatgccctctggggaggggaaagaggaggggaggaggatgaagaggggcaagaggagctccctgcccagcccagccagcaagcctggagaagcacttgctagagctaaggaagcctcggagctggacgggtgccccccacccctcatcataacctgaagaacatggaggcccgggaggggtgtcacttgcccaaagctacacagggggtggggctggaagtggctccaagtgcaggttcccccctcattcttcaggcttagggctggaggaagccttagacagcccagtcctaccccagacagggaaactgaggcctggagagggccagaaatcaccctgacctcttctcttcctcccacagatgcagcgcgtgaacatgatcatggccgagtctcctggcctgatcaccatctgcctgctgggctacctgctgagcgccgagtgcaccgtgtttctggaccacgagaacgccaacaagatcctgaaccggcccaagcggtacaacagcggcaagctggaagagttcgtgcagggcaacctggaacgcgagtgcatggaagagaagtgcagctttgaagaggccagagaggtgttcgagaacaccgagcggaccaccgagttctggaagcagtatgttgatggagatcagtgtgagtccaatccatgtttaaatggcggcagttgcaaggatgacattaattcctatgaatgttggtgtccctttggcttcgagggcaagaactgtgaattagatgtaacatgtaacattaagaatggcagatgcgagcagttttgtaaaaatagtgctgataacaaggtggtttgctcctgtactgagggatatcgacttgcagaaaaccagaagtcctgcgagcccgccgtgcctttcccatgtggaagagtgtccgtgtcccagaccagcaagctgaccagagccgagacagtgttccccgacgtggactacgtgaacagcaccgaggccgagacaatcctggacaacatcacccagagcacccagtccttcaacgacttcaccagagtcgtgggcggcgaggatgccaagcctggacagttcccgtggcaggtggtgctgaacggaaaggtggacgccttttgcggcggcagcatcgtgaatgaaaaatggattgtaactgctgcccactgtgttgaaactggtgttaaaattacagttgtcgcaggtgaacataacatcgaggaaaccgaacatacagagcaaaagcgaaatgtgattcgaattattcctcaccacaactacaatgcagctattaataagtacaaccatgacattgcccttctggaactggacgaacccttagtgctaaacagctacgttacacctatttgcattgctgacaaagagtacaccaacatctttctgaagttcggcagcggctacgtgtccggctggggcagagtgtttcacaagggcagatccgctctggtgctgcagtacctgagagtgcctctggtggaccgggccacctgtctgagaagcaccaagttcaccatctacaacaacatgttctgcgccggctttcacgagggcggcagagatagctgtcagggcgattctggcggccctcacgtgacagaggtggaaggcaccagctttctgaccggcatcatcagctggggcgaggaatgcgccatgaaggggaagtacggcatctacaccaaggtgtccagatacgtgaactggatcaaagaaaagaccaagctgacatgactgtgccttctagttgccagccatctgttgtttgcccctcccccgtgccttccttgaccctggaaggtgccactcccactgtcctttcctaataaaatgaggaaattgcatcgcattgtctgagtaggtgtcattctattctggggggtggggtggggcaggacagcaagggggaggattgggaagacaatagcaggcatgctggggatgcggtgggctctatgg

SEQ ID NO: 38 - DNA, 2511 bp, synthetic construct
  source 1..2511: mol_type = other DNA
atgcagcgcgtgaacatgatcatggccgagtctcctggcctgatcaccatctgcctgctgggctacctgctgagcgccgagtgcaccgtgtttctggaccacgagaacgccaacaagatcctgaaccggcccaagcggtacaacagcggcaagctggaagagttcgtgcagggcaacctggaacgcgagtgcatggaagagaagtgcagctttgaagaggccagagaggtgttcgagaacaccgagcggaccaccgagttctggaagcagtatgttgatggagatcagtgtgagtccaatccatgtttaaatggcggcagttgcaaggatgacattaattcctatgaatgttggtgtccctttggcttcgagggcaagaactgtgaattagatgtaacatgtaacattaagaatggcagatgcgagcagttttgtaaaaatagtgctgataacaaggtggtttgctcctgtactgagggatatcgacttgcagaaaaccagaagtcctgcgagcccgccgtgcctttcccatgtggaagagtgtccgtgtcccagaccagcaagctgaccagagccgagacagtgttccccgacgtggactacgtgaacagcaccgaggccgagacaatcctggacaacatcacccagagcacccagtccttcaacgacttcaccagagtcgtgggcggcgaggatgccaagcctggacagttcccgtggcaggtggtgctgaacggaaaggtggacgccttttgcggcggcagcatcgtgaatgaaaaatggattgtaactgctgcccactgtgttgaaactggtgttaaaattacagttgtcgcaggtgaacataacatcgaggaaaccgaacatacagagcaaaagcgaaatgtgattcgaattattcctcaccacaactacaatgcagctattaataagtacaaccatgacattgcccttctggaactggacgaacccttagtgctaaacagctacgttacacctatttgcattgctgacaaagagtacaccaacatctttctgaagttcggcagcggctacgtgtccggctggggcagagtgtttcacaagggcagatccgctctggtgctgcagtacctgagagtgcctctggtggaccgggccacctgtctgagaagcaccaagttcaccatctacaacaacatgttctgcgccggctttcacgagggcggcagagatagctgtcagggcgattctggcggccctcacgtgacagaggtggaaggcaccagctttctgaccggcatcatcagctggggcgaggaatgcgccatgaaggggaagtacggcatctacaccaaggtgtccagatacgtgaactggatcaaagaaaagaccaagctgacatgactgtgccttctagttgccagccatctgttgtttgcccctcccccgtgccttccttgaccctggaaggtgccactcccactgtcctttcctaataaaatgaggaaattgcatcgcattgtctgagtaggtgtcattctattctggggggtggggtggggcaggacagcaagggggaggattgggaagacaatagcaggcatgctggggatgcggtgggctctatggcaaagacacacagcatgttggctggactggacggagatcagtccagaccgcaggtgccttgatgttcagtctggtgggttttctgctccatcccacccacctccctttgggcctcgatccctcgcccctcaccagtcccccttctgagagcccgtattagcagggagccggcccctactccttctggcagacccagctaaggttctaccttaggggccacgccacctccccagggaggggtccagaggcatggggacctggggtgcccctcacaggacacttccttgcaggaacagaggtgccatgcagccccgggtactccttgttgttgccctcctggcgctcctggcctctgcccgtaagcacttggtgggactgggctgggggcagggtggaggcaacttggggatcccagtcccaatgggtggtcaagcaggagcccagggctcgtccagaggccgatccaccccactcagccctgctctttcctcaggagcttcagaggccgaggatgcctcccttctcagcttcatgcagggttacatgaagcacgccaccaagaccgccaaggatgcactgagcagcgtgcaggagtcccaggtggcccagcaggccaggtacacccgctggcctccctccccatcccccctgccagctgcctccattcccacccgcccctgccctggtgagatcccaacaatggaatggaggtgctccagcctcccctgggcctgtgcctcttcagcctcctctttcctcacagggcctttgtcaggctgctgcgggagagatgacagagttgagactgcattcctcccaggtccctcctttctccccggagcagtcctagggcgtgccgttttagccctcatttccattttcctttcctttccctttctt

SEQ ID NO: 39 - DNA, 3636 bp, synthetic construct
  source 1..3636: mol_type = other DNA
tgcccagctacggcagaggagactgttgggatcacaggtggaggtcagtgtgggggcatgtaaccttcactctgccccctcccaccccacttcctccgttgctccacagtggcaccacagattccccattccattctactggaaggctttcaggtggcttctgtgaaggagcctgtcactggctctaggctgtaaagcaggcctgaggtccaaggcttgtcccctgtcttttcctgtctcaccgacctcatctaggtgagccggtagctgatcccttggtggcggaggtggccgtgaaaagcatgggcaatctcagagggatttctcaactcctctggcagatggctgcatggccttcctgcctcaggctctggtctggactgctcagcaggtgacctttgcccagctcactgggccttctgtgcccgctgtcccatcctggagccaatataaaacaggtcacagccctccccgcttgcctgctcagttttatccctagaagcagctagctactccaggtaatgcccctggggaggagaggaaggaagggaagaaacaaagagctggagggagaagctctcaccacccagccatctagcccacagaaggcttgggactcatggtctccacccttgggttcctggtgtggggggggctagaagctggggaaagggaggctatgggccaaaagccttgcactgggtagtggcagagctgcctgcaattgggtcatgctgtcccttgtttagcttgctctgagctattagaagcctttggtatccatgcctacccaggactgaaaaaactgagtcctagcgaggaaaagaaacctattgtttctcagcatattagagtagatgtcccgttctgcagagtatttctatactccaccttccaggttcccccctcattcttcaggcttagggctggaggaagccttagacagcccagtcctaccccagacagggaaactgaggcctggagagggccagaaatcaccctgacctcttctcttcctcccacagatgcagcgcgtgaacatgatcatggccgagtctcctggcctgatcaccatctgcctgctgggctacctgctgagcgccgagtgcaccgtgtttctggaccacgagaacgccaacaagatcctgaaccggcccaagcggtacaacagcggcaagctggaagagttcgtgcagggcaacctggaacgcgagtgcatggaagagaagtgcagctttgaagaggccagagaggtgttcgagaacaccgagcggaccaccgagttctggaagcagtatgttgatggagatcagtgtgagtccaatccatgtttaaatggcggcagttgcaaggatgacattaattcctatgaatgttggtgtccctttggcttcgagggcaagaactgtgaattagatgtaacatgtaacattaagaatggcagatgcgagcagttttgtaaaaatagtgctgataacaaggtggtttgctcctgtactgagggatatcgacttgcagaaaaccagaagtcctgcgagcccgccgtgcctttcccatgtggaagagtgtccgtgtcccagaccagcaagctgaccagagccgagacagtgttccccgacgtggactacgtgaacagcaccgaggccgagacaatcctggacaacatcacccagagcacccagtccttcaacgacttcaccagagtcgtgggcggcgaggatgccaagcctggacagttcccgtggcaggtggtgctgaacggaaaggtggacgccttttgcggcggcagcatcgtgaatgaaaaatggattgtaactgctgcccactgtgttgaaactggtgttaaaattacagttgtcgcaggtgaacataacatcgaggaaaccgaacatacagagcaaaagcgaaatgtgattcgaattattcctcaccacaactacaatgcagctattaataagtacaaccatgacattgcccttctggaactggacgaacccttagtgctaaacagctacgttacacctatttgcattgctgacaaagagtacaccaacatctttctgaagttcggcagcggctacgtgtccggctggggcagagtgtttcacaagggcagatccgctctggtgctgcagtacctgagagtgcctctggtggaccgggccacctgtctgagaagcaccaagttcaccatctacaacaacatgttctgcgccggctttcacgagggcggcagagatagctgtcagggcgattctggcggccctcacgtgacagaggtggaaggcaccagctttctgaccggcatcatcagctggggcgaggaatgcgccatgaaggggaagtacggcatctacaccaaggtgtccagatacgtgaactggatcaaagaaaagaccaagctgacatgactgtgccttctagttgccagccatctgttgtttgcccctcccccgtgccttccttgaccctggaaggtgccactcccactgtcctttcctaataaaatgaggaaattgcatcgcattgtctgagtaggtgtcattctattctggggggtggggtggggcaggacagcaagggggaggattgggaagacaatagcaggcatgctggggatgcggtgggctctatggcaaagacacacagaccacttggggggctgggtctactgtagttctctatctaatatcagtgggagaaaggcttgggattcatgacccaggagtcatggcattctcaaggggaggacctagatgtggcagatccacagtaccttctcacgagatgctttcccacaggtacgtaggtgccatgcagccccggacgctcctcactgtggccctcttggctctcctggcatctgcccgtaagatggtgggagtggggctgggtttcagtgggagctggtcagggggccctgccctgagaagtggtggctgggcaggagctgagggctggcgtggcccaactctgctctctcgcaggagctgaagaggtagagggatccttgctgctgggctctgtacagggctacatggaacaagcctccaagacggtccaggatgcgctaagtagcgtgcaggagtccgatatagctgtggtggccaggtaggcacactggcctcctttcctgtgtcttctcctctcatgccctggtgctaagaccctagcacagagactgtggtccaccaagtttaccagggcctgggacccgcccgagcctctggtccctcatgaggcctttcggtactgtgaccaagatgacaggcagggcaagcagccttctcctatcttctctgcttttcctcagagcagcctgaggggcatttagcctcgctgcaggttttctcctctgggtcctgcgcacacgatgggaggcctacctgctctggtttctgcctgtatgcagggggtagtggtgggaagtgaggtgggaagttgggggttagagggtgggagtctgccctgtttctatccctgggctcagtctgaggtaggcatcttgcccactatgaaatatcaccccctggccaatggctttggctgacatttgatagtttagttgcctatgtagcaaaagatgttgacagtctctatccccagaacaggctgtggggaggatattagatactc

SEQ ID NO: 40 - DNA, 22 bp, synthetic construct
  source 1..22: mol_type = other DNA
gagagggccagaaatcacccaa